European Patent Application EP 4 772 024 A1, published July 8, 2026. Title: OFF-FLAVOR-SUPPRESSING MATERIAL, FLAVOR COMPOSITION FOR SUPRESSING OFF-FLAVOR, AND FOOD AND DRINK IN WHICH OFF-FLAVOR CONTAINED IN THE FOOD AND DRINK IS MASKED. Applicant: 高砂香料工業株式会社. The sequence listing filed with the application follows.

SEQUENCE LISTING (4 sequences)

SEQ ID NO: 1 - DNA, 4224 bp, Homo sapiens
  source 1..4224: mol_type = genomic DNA
  CDS 893..1843: protein_id = 2; translation = MELRNSTLGSGFILVGILNDSGSPELLYATFTILYMLALTSNGLLLLAITIEARLHMPMYLLLGQLSLMDLLFTSVVTPKALADFLRRENTISFGGCALQMFLALTMGSAEDLLLAFMAYDRYVAICHPLKYMTLMSPRVCWIMVATSWILASLIAIGHTMYTMHLPFCVSWEIRHLLCEIPPLLKLACADTSRYELIIYVTGVTFLLLPISAIVASYTLVLFTVLRMPSNEGRKKALVTCSSHLIVVGMFYGAATFMYVLPSSFHSPKQDNIISVFYTIVTPALNPLIYSLRNKEVMRALRRVLGKYILLAHSTL
atgaaacacagcatgaggggaatatatgaaatctgaggacctggacttaagaactcagctagaaccattccaaagcagtaaggactttctcgcaaggacagtgaatgagagaactttggaagagattcagctcctcacttctgcaggatcctgccctaggttctcagctgcctgtctgcatctatctctacttccagagaggacttgcagtgccagtgactggaggagcctttgatctctgatcctagagacagccatacacacacctacattcatcctggccagaagaagcaacttttctttctttggcttcttgaacctctttacctggaagctatgccccttcccatatgagcagagcagcacttgaagagtccaggtgatcaagcagcccaagaacccagagattctcctactgaggaaagtaatcaacaacaatgagactggtttaagggagaagacagcaaagaggttttttataaataaaattttaaaaactgaattggaattccaactacattttaagcagaaaaatagctagatcttaaaccaatccccagtatatttgttcattgtgaagaaagagatgctttcatctatctacaaagatgtttgcttgggcttattcttcaggataccttatttgaagggatttctaaatgattactattaacaacatgtcaaaatacctgataccagtttagctgatggtttatttcaataaaagcattcagaaatcagaggcatactaagaaatggaaaatatatcatattatgggattcctattggccaatgcacagtgacctagaacaatccaaagctagagtgaacacctttagaaaagcttccactgataatatatttggttctaggcaactaaaaaaacacatcatggagctccggaactccaccttgggaagcggcttcatcttggtggggattctgaatgacagtgggtctcctgaactgctctatgctacatttacaatcctatacatgttggcactgaccagcaatggtctgctgctcctggccatcaccatagaagcccggctccacatgcccatgtacctcctgcttgggcagctctctctcatggacctcctgttcacatctgttgtcactcccaaggcccttgcggactttctgcgcagagaaaacactatctcctttggaggctgtgcacttcagatgttcctggcactgacaatgggtagcgctgaggacctcctactggccttcatggcctatgacaggtatgtggccatttgtcatcctctgaaatacatgaccctcatgagcccaagagtctgctggatcatggtggccacatcctggatcctggcatccctgattgctataggacataccatgtacactatgcacctccctttctgtgtgtcctgggaaatcaggcatctgctctgtgagatcccacccttgctgaagttggcctgtgctgatacctccaggtatgagcttataatatacgtgacaggtgtgactttcctcttgctccccatttctgccattgtggcctcctacacactagtcctattcactgtgcttcgtatgccatcaaatgaggggaggaagaaagcccttgtcacctgctcttcccacctgattgtggtcgggatgttctatggagctgccacattcatgtatgtcttgcccagttccttccacagccccaaacaagacaacatcatctctgttttctacacaattgtcactccagccctgaatccactcatctacagcctgaggaataaggaggtcatgcgggccttgaggagggtcctgggaaaatacatactgctggcacattccacgctctagggaaggatcatggcttgcctctcaccattcctcctccagataaaattctctactcactcattcctgctccaaataaaattctctactcactcattcttcaatactgtactctgagatgatagatacattttttaaattttacttttattttcaactgtgaatctggtgtgtacaatgatcttgagttaaactcatttggcacacatcatcctgactttggaaacccatgttataaaaataaccagatgggggaaaagccttgaatgggtgttgtagactcactctgtggtaggcatcgtcctgacacattaccaagtagacatggtaggggattagctttccattttaacatcacatagcagtgagaagcagcagtagttttggactgaccaaattccaatagcctctcagcatcagaggaggactactccctttgaagcagattcttaaactactaatagagggaagaattttcagaagatatattagacttcctgtttattaagtagatgattatttgagcagttagtggaaatgaataagagttatgtgactgcatttgtactctagacctaagggaccttcacattggttacttgagtaatgataaataattacattgaaagagtgtggccaggcgcagtagctcacgcctgtaatccaagcactttgggaggctgaggtgggcagatcacctgaggtaaggagttcaagaccagcctggccaacgtgtggaacccgggtctctactaaaaatacaaaaatgagcggggcatagttgtgggtgcctgtaatcccagctactcgggaggctgaggcaggagaattgcttgaccctgggaggcggaggtcgcagtgagctgagatcgcgccactgcactccagcctgagcaacagagagagactccgtttcaataaataaataaataaatagaaagaaagaatggaaaaggataaagaaagatatttctacttggaaattttgacagtctttttgaaaatgggcatttttacattgcctaaaattaaaactaaaataaagaatgaataaaatagaattgaaagtaccagttttaaagtgagtacaataacaatgagagaaatttgttgggaatattgtctaagttttttaaaatgtggacttgcagatatgtgaatgtgtttttaaacattaaaacaattgaaagaggttatattcttgaggtgagtgtatgtacatgtgtgtttccatagaaaaggaagtataaaatttataatttgctttctagctagcctaaataagccttattttttttattctactcatcagtgtgggaagatttatagcaaaatttgggaacttaaatttgttgaatgcagaattcccaaaatatcttggcttacataggtgttattattcttgagaatagtgctttgtcaaaacacaataattcttgttttctttatagaaataatattacattatttaatctataaagctaaaccataaaaaataaaagataaagctaatctataaaattaatccaactttgttataaaaactgagaaaattaaaaaaattagaataaatcaaaaatcacttataaatttttcttttttgttgcacatatatgcattttactgaatttaaatgtccatgatgatgaaggtcctgtgttttttccatttgaaatttggtgaatcttcttccttgctatgagggaatattttagagtagtgatgagaaagcagaccagagtgcccgcatttgaatccctctcttcctttggtcatctatgcatctttgaacgctaaattaaactctttgtaccttagtctgctgatgttaaaagtggtgatatttactggcctgctcttgtgatattgttgggtagattaaataagataattaatatcaggtactgagaccacagcttagtaaactgtgcttaaaacattttggctgctatatggataaatagtaaaaagcctttttaaaaaatcttattttattatttccttttagaaatgaaacatttgtttattatttttattgacaaaatatgtatgtcttaatgtagtaaaacatgatgttttgaaatatgtatactttatggaattgctaaatcaagccaactaacatatgctttactccacatacttatcttttttgcattaggaaaagttaaaatctactttctcagcaattttcaagcacacaatataatctgattaactataattgccatgatctacaataaatctcttgaacttattcctcctgtctaactgaagttttgtgtcctttcaccagcatctcccaaatccccctacctcaacatttggtaaccaccattttactctctgtttctgtaaattcagcttacaggttctgcatataa

SEQ ID NO: 2 - protein, 316 aa, Homo sapiens
MELRNSTLGSGFILVGILNDSGSPELLYATFTILYMLALTSNGLLLLAITIEARLHMPMYLLLGQLSLMDLLFTSVVTPKALADFLRRENTISFGGCALQMFLALTMGSAEDLLLAFMAYDRYVAICHPLKYMTLMSPRVCWIMVATSWILASLIAIGHTMYTMHLPFCVSWEIRHLLCEIPPLLKLACADTSRYELIIYVTGVTFLLLPISAIVASYTLVLFTVLRMPSNEGRKKALVTCSSHLIVVGMFYGAATFMYVLPSSFHSPKQDNIISVFYTIVTPALNPLIYSLRNKEVMRALRRVLGKYILLAHSTL

SEQ ID NO: 3 - DNA, 2445 bp, Bos taurus
  source 1..2445: mol_type = genomic DNA
  CDS 1..1047: protein_id = 4; translation = MNGTEGPNFYVPFSNKTGVVRSPFEAPQYYLAEPWQFSMLAAYMFLLIMLGFPINFLTLYVTVQHKKLRTPLNYILLNLAVADLFMVFGGFTTTLYTSLHGYFVFGPTGCNLEGFFATLGGEIALWSLVVLAIERYVVVCKPMSNFRFGENHAIMGVAFTWVMALACAAPPLVGWSRYIPEGMQCSCGIDYYTPHEETNNESFVIYMFVVHFIIPLIVIFFCYGQLVFTVKEAAAQQQESATTQKAEKEVTRMVIIMVIAFLICWLPYAGVAFYIFTHQGSDFGPIFMTIPAFFAKTSAVYNPVIYIMMNKQFRNCMVTTLCCGKNPLGDDEASTTVSKTETSQVAPA
atgaacgggaccgagggcccaaacttctacgtgcctttctccaacaagacgggcgtggtgcgcagccccttcgaggccccgcagtactacctggcggagccatggcagttctccatgctggccgcctacatgttcctgctgatcatgcttggcttccccatcaacttcctcacgctgtacgtcacagtccagcacaagaagctgcgcacacccctcaactacatcctgctcaacctggccgtggccgacctcttcatggtcttcgggggcttcaccaccaccctctacacctctctgcacggatacttcgtctttgggcccacgggctgcaacctggagggcttctttgccaccctgggcggtgaaattgcactgtggtccttggtggtcctggccatcgagcggtacgtggtggtgtgcaagcccatgagcaacttccgcttcggggagaaccacgccatcatgggcgtcgccttcacctgggtcatggctctggcctgtgccgcgccccccctcgtcggctggtccaggtacatcccggagggcatgcagtgctcgtgcgggattgactactacacgccccacgaggagaccaacaatgagtcgttcgtcatctacatgttcgtggtccacttcatcatccccctgattgtcatattcttctgctacgggcagctggtgttcaccgtcaaggaggcggctgcccagcagcaggagtcggccaccactcagaaggccgagaaggaggtcacccgcatggtgatcatcatggtcatcgctttcctaatctgctggctgccctacgctggggtggcgttctacatcttcacccatcagggctctgactttggccccatcttcatgaccatcccggctttctttgccaagacttctgccgtctacaaccccgtcatctacatcatgatgaacaagcagttccggaactgcatggtcaccactctctgctgtggcaagaacccgctgggtgacgacgaggcctccaccaccgtctccaagacagagaccagccaggtggcgcctgcctaagcccctccagggactccgtggccagctgcaggagtccctcagcccccaccccaccccagcctcagcagctccatcaggagccgcgcctgtcggaaccagctctcacaggctccctgagtgtaaacacaaagaccaaccaaccaaatgcaaaagaatcaacgagagaaacaggaggcgcctcacgtggcaggggcggcccgatctggagtcctgatttcccgggggcccgctgtagatccactccccccagctcatctctcagctacacaagagctcttgctctggaaaagtgtcccagcttagggataagtgagtagcacatgacggggcatgccgtaggtgcttattaataaatgctaggtggaggaaagaaggaatgaatggagagatgaacgggtcgggagggcataggcatcctcttacaacatgttagcagcagcagcagcagctcgcccttggctcatgaccttgagcagctgttttgtccttgggcctcactttcttcccccatacaatgggaattccaaatctctcctcacacgggctgctgggaagatcaaatgagattgtgtgtgtgtgcgtgcgtgcgtgctcgcttgtgtgagctctttgtaaatagtaaggagctggacagactgtagttaacattatgaataatatcaagtaatataagtaattcatctcctatgatcatctcctcttgatagcgaccactttgagactgggcaaggctctaagcatccagcctcgtcaggcttataaacattagacagatggcaaggtcagaccagcgccgggtggtgggccacagggaaggacggtcaaggaaatgcagagtgcaggcatcaggcctgagaagaaaacaaaaaccaaaaaaacaacatcagaggaccagagtctggggccagtgcagagcccccatgacgcgggccactccctcccagtgcaacccccagagagacaggtcttgctctcggcatctgaaaaaccactagctctcctgcccagcacccaggctgcagtatctctgggcccgtatggagcttctagaagttatgtttacctgcccacatttaacgaagagctgggtccccaacatcacctttgtctcaaaaagagcttaaaaaacaaaagcgtgggaaatccggctggacccaccttccccctgggaagttcacagatcacagattttagctcccttgctgggcaagccttcagcggctccagtccattctccactccggagagtccttgctgctgagaggctggctgggactctaggacatcagaatcgagccgcctcataactgcccctcctccactacataaccaaagcgggaagctctacctctccccagctctgcctggagacgaaggcaaattggggtattaaaagct

SEQ ID NO: 4 - protein, 348 aa, Bos taurus
MNGTEGPNFYVPFSNKTGVVRSPFEAPQYYLAEPWQFSMLAAYMFLLIMLGFPINFLTLYVTVQHKKLRTPLNYILLNLAVADLFMVFGGFTTTLYTSLHGYFVFGPTGCNLEGFFATLGGEIALWSLVVLAIERYVVVCKPMSNFRFGENHAIMGVAFTWVMALACAAPPLVGWSRYIPEGMQCSCGIDYYTPHEETNNESFVIYMFVVHFIIPLIVIFFCYGQLVFTVKEAAAQQQESATTQKAEKEVTRMVIIMVIAFLICWLPYAGVAFYIFTHQGSDFGPIFMTIPAFFAKTSAVYNPVIYIMMNKQFRNCMVTTLCCGKNPLGDDEASTTVSKTETSQVAPA